European Patent Application EP 4 428 225 A1, published September 11, 2024. Title: Engineered obligate fermenting bacteriaEscherichia coli strain for the fermentative production of D-lactate. Applicant: Max-Planck-Gesellschaft zur Foerderung der Wissenschaften e.V. The sequence listing filed with the application follows.

SEQUENCE LISTING (94 sequences)

SEQ ID NO: 1 - DNA, 72 bp, Escherichia coli
  source 1..72: mol_type = other DNA
taataaccattaattaacaattggttaataaatttaagggggtcacgttgaattaaccctcactaaagggcg

SEQ ID NO: 2 - DNA, 73 bp, Escherichia coli
  source 1..73: mol_type = other DNA
tttatgccacatccgccagtgtacgtcgattaatgcaacttcaaacgcggtaatacgactcactatagggctc

SEQ ID NO: 3 - DNA, 23 bp, Escherichia coli
  source 1..23: mol_type = other DNA
gcgaagaacattttcattgctgt

SEQ ID NO: 4 - DNA, 20 bp, Escherichia coli
  source 1..20: mol_type = other DNA
aggatgcctgatacaacgcg

SEQ ID NO: 5 - DNA, 20 bp, Escherichia coli
  source 1..20: mol_type = other DNA
ggttacccatcaggctaccg

SEQ ID NO: 6 - DNA, 20 bp, Escherichia coli
  source 1..20: mol_type = other DNA
cacagctggggcataagctg

SEQ ID NO: 7 - DNA, 70 bp, Escherichia coli
  source 1..70: mol_type = other DNA
gatctcaatcagttccggtgatatccaactcattgttgtgcctccttgaggtgtaggctggagctgcttc

SEQ ID NO: 8 - DNA, 70 bp, Escherichia coli
  source 1..70: mol_type = other DNA
tatctgggcagtatcgattttgttatgtcagatgtggaccgctaattatgcatatgaatatcctccttag

SEQ ID NO: 9 - DNA, 26 bp, Escherichia coli
  source 1..26: mol_type = other DNA
cggtgccagggtaaagatgacgcgat

SEQ ID NO: 10 - DNA, 26 bp, Escherichia coli
  source 1..26: mol_type = other DNA
tcgaaaccctgatcacccacttcctg

SEQ ID NO: 11 - DNA, 20 bp, Escherichia coli
  source 1..20: mol_type = other DNA
cgatcgagcacgagatgcac

SEQ ID NO: 12 - DNA, 20 bp, Escherichia coli
  source 1..20: mol_type = other DNA
cgatttcaaccggcagcgtg

SEQ ID NO: 13 - DNA, 70 bp, Escherichia coli
  source 1..70: mol_type = other DNA
cttttctgcgatacaatgcctttacgttatgtaacggagagttcggcatggtgtaggctggagctgcttc

SEQ ID NO: 14 - DNA, 70 bp, Escherichia coli
  source 1..70: mol_type = other DNA
ccggatgatcatccggcttttttacatcatcagaaatgccagtaactcatcatatgaatatcctccttag

SEQ ID NO: 15 - DNA, 22 bp, Escherichia coli
  source 1..22: mol_type = other DNA
ttttactgcgagttggcgagct

SEQ ID NO: 16 - DNA, 22 bp, Escherichia coli
  source 1..22: mol_type = other DNA
gcagggcgaagggtaatcagag

SEQ ID NO: 17 - DNA, 18 bp, Escherichia coli
  source 1..18: mol_type = other DNA
gctggcggcgatcaaaga

SEQ ID NO: 18 - DNA, 29 bp, Escherichia coli
  source 1..29: mol_type = other DNA
gcggttgcacctttcaaaaatgttaactg

SEQ ID NO: 19 - DNA, 20 bp, Escherichia coli
  source 1..20: mol_type = other DNA
gcagcggtattcacactcag

SEQ ID NO: 20 - DNA, 20 bp, Escherichia coli
  source 1..20: mol_type = other DNA
cacaccagccattcctcgac

SEQ ID NO: 21 - DNA, 70 bp, Escherichia coli
  source 1..70: mol_type = other DNA
gaatgactttagttttcattttgttattccttttcaagggcttgttctacgtgtaggctggagctgcttc

SEQ ID NO: 22 - DNA, 72 bp, Escherichia coli
  source 1..72: mol_type = other DNA
cgcgcaaaaatcagctgccacacaacacaacaaagcgaagcctactcatgggaattagccatggtccatatg

SEQ ID NO: 23 - DNA, 22 bp, Escherichia coli
  source 1..22: mol_type = other DNA
cgcagtcacgaacgcggtacgt

SEQ ID NO: 24 - DNA, 25 bp, Escherichia coli
  source 1..25: mol_type = other DNA
cacacagtcgacgttccgagggaag

SEQ ID NO: 25 - DNA, 20 bp, Escherichia coli
  source 1..20: mol_type = other DNA
ggataacctgtcgatccgcg

SEQ ID NO: 26 - DNA, 20 bp, Escherichia coli
  source 1..20: mol_type = other DNA
gtgacgcacagaggtacgac

SEQ ID NO: 27 - DNA, 22 bp, Escherichia coli
  source 1..22: mol_type = other DNA
ttcttcctttgttgcccgacgt

SEQ ID NO: 28 - DNA, 22 bp, Escherichia coli
  source 1..22: mol_type = other DNA
tagtgatggacgcgtttggcaa

SEQ ID NO: 29 - DNA, 20 bp, Escherichia coli
  source 1..20: mol_type = other DNA
gaacttgctcgtctggtggg

SEQ ID NO: 30 - DNA, 20 bp, Escherichia coli
  source 1..20: mol_type = other DNA
gaacttgctcgtctggtggg

SEQ ID NO: 31 - DNA, 20 bp, Escherichia coli
  source 1..20: mol_type = other DNA
gccgcatccaacatctaacg

SEQ ID NO: 32 - DNA, 16 bp, Escherichia coli
  source 1..16: mol_type = other DNA
cggactgctgccgtca

SEQ ID NO: 33 - DNA, 20 bp, Escherichia coli
  source 1..20: mol_type = other DNA
cggtttcaactgcggtttcg

SEQ ID NO: 34 - DNA, 20 bp, Escherichia coli
  source 1..20: mol_type = other DNA
ggaactgaactacaccccgc

SEQ ID NO: 35 - DNA, 25 bp, Escherichia coli
  source 1..25: mol_type = other DNA
gacgccatattgccgcagagtcagg

SEQ ID NO: 36 - DNA, 21 bp, Escherichia coli
  source 1..21: mol_type = other DNA
gtcgcggcctggcggacaatg

SEQ ID NO: 37 - DNA, 21 bp, Escherichia coli
  source 1..21: mol_type = other DNA
cattgggtaactgcaggccgc

SEQ ID NO: 38 - DNA, 25 bp, Escherichia coli
  source 1..25: mol_type = other DNA
cgagttgtcatactgggaagtggtg

SEQ ID NO: 39 - DNA, 20 bp, Escherichia coli
  source 1..20: mol_type = other DNA
agtgcctcctttctctccca

SEQ ID NO: 40 - DNA, 20 bp, Escherichia coli
  source 1..20: mol_type = other DNA
gtcgtctccgtaaacgtcgt

SEQ ID NO: 41 - DNA, 21 bp, Escherichia coli
  source 1..21: mol_type = other DNA
ggttaatcggcttctcgtcag

SEQ ID NO: 42 - DNA, 20 bp, Escherichia coli
  source 1..20: mol_type = other DNA
gaacttgctcgtctggtggg

SEQ ID NO: 43 - DNA, 25 bp, Escherichia coli
  source 1..25: mol_type = other DNA
cagcaatatgacgatccgcgggcag

SEQ ID NO: 44 - DNA, 30 bp, Escherichia coli
  source 1..30: mol_type = other DNA
ctcggcaaagtgcagaatagattcggcatc

SEQ ID NO: 45 - DNA, 20 bp, Escherichia coli
  source 1..20: mol_type = other DNA
ctcctgccattccagcagac

SEQ ID NO: 46 - DNA, 20 bp, Escherichia coli
  source 1..20: mol_type = other DNA
gcatccgtatccgcatcatt

SEQ ID NO: 47 - DNA, 26 bp, Escherichia coli
  source 1..26: mol_type = other DNA
gtcgtacccggcgacttcgaaaatgg

SEQ ID NO: 48 - DNA, 37 bp, Escherichia coli
  source 1..37: mol_type = other DNA
ggttgtgaaatttgcactctgaaaaggacgtcttatc

SEQ ID NO: 49 - DNA, 21 bp, Escherichia coli
  source 1..21: mol_type = other DNA
catattgaaacgatggcacgc

SEQ ID NO: 50 - DNA, 20 bp, Escherichia coli
  source 1..20: mol_type = other DNA
caatagacagttcttcctgg

SEQ ID NO: 51 - DNA, 22 bp, Escherichia coli
  source 1..22: mol_type = other DNA
aggcggtacttatactcccgca

SEQ ID NO: 52 - DNA, 22 bp, Escherichia coli
  source 1..22: mol_type = other DNA
aaaagcgagaagtacgggcagg

SEQ ID NO: 53 - DNA, 20 bp, Escherichia coli
  source 1..20: mol_type = other DNA
gctttctgatgtctcgatgg

SEQ ID NO: 54 - DNA, 20 bp, Escherichia coli
  source 1..20: mol_type = other DNA
ctttctccggcaactttacc

SEQ ID NO: 55 - DNA, 27 bp, Escherichia coli
  source 1..27: mol_type = other DNA
cggatattcacagccgcgccaacaatc

SEQ ID NO: 56 - DNA, 31 bp, Escherichia coli
  source 1..31: mol_type = other DNA
gtgcgtaatcatcgttgcgctgctgtttatc

SEQ ID NO: 57 - DNA, 20 bp, Escherichia coli
  source 1..20: mol_type = other DNA
caccaaatgcggtcaattgc

SEQ ID NO: 58 - DNA, 21 bp, Escherichia coli
  source 1..21: mol_type = other DNA
catttaatggcatggttgcac

SEQ ID NO: 59 - DNA, 70 bp, Escherichia coli
  source 1..70: mol_type = other DNA
gtcaggatggccgggcaaacaaggcaggattaaatccctggctgcagaatcatatgaatatcctccttag

SEQ ID NO: 60 - DNA, 29 bp, Escherichia coli
  source 1..29: mol_type = other DNA
cctgcatcggtgagtcagagtaagatcag

SEQ ID NO: 61 - DNA, 29 bp, Escherichia coli
  source 1..29: mol_type = other DNA
cctgcatcggtgagtcagagtaagatcag

SEQ ID NO: 62 - DNA, 26 bp, Escherichia coli
  source 1..26: mol_type = other DNA
ggttgcaagagaaaggcgacatggcg

SEQ ID NO: 63 - DNA, 21 bp, Escherichia coli
  source 1..21: mol_type = other DNA
gtatagcggggaacatcaggc

SEQ ID NO: 64 - DNA, 20 bp, Escherichia coli
  source 1..20: mol_type = other DNA
cgcccactccaatggtcaac

SEQ ID NO: 65 - DNA, 22 bp, Escherichia coli
  source 1..22: mol_type = other DNA
accgcctctttttcctgcaact

SEQ ID NO: 66 - DNA, 22 bp, Escherichia coli
  source 1..22: mol_type = other DNA
aatttttatgctggcgctgggc

SEQ ID NO: 67 - DNA, 20 bp, Escherichia coli
  source 1..20: mol_type = other DNA
gatagggggcggcatcaatg

SEQ ID NO: 68 - DNA, 20 bp, Escherichia coli
  source 1..20: mol_type = other DNA
cggcaccacaatatggctgc

SEQ ID NO: 69 - DNA, 22 bp, Escherichia coli
  source 1..22: mol_type = other DNA
catgcgcggtttcttcgatgtc

SEQ ID NO: 70 - DNA, 22 bp, Escherichia coli
  source 1..22: mol_type = other DNA
tgcggtgtcgtttcagagtgag

SEQ ID NO: 71 - DNA, 20 bp, Escherichia coli
  source 1..20: mol_type = other DNA
gcattgcaggtgtggatcgt

SEQ ID NO: 72 - DNA, 20 bp, Escherichia coli
  source 1..20: mol_type = other DNA
cactatatggatggtggtgc

SEQ ID NO: 73 - DNA, 70 bp, Escherichia coli
  source 1..70: mol_type = other DNA
tttttactatggctaaatggtaaaaaacgaacttcagagggataacaatggtgtaggctggagctgcttc

SEQ ID NO: 74 - DNA, 70 bp, Escherichia coli
  source 1..70: mol_type = other DNA
cacatgcttaccgggcatcagaaaggagtttaagccagcgcctgggccagcatatgaatatcctccttag

SEQ ID NO: 75 - DNA, 22 bp, Escherichia coli
  source 1..22: mol_type = other DNA
cgtttcttgagttgccgcgatg

SEQ ID NO: 76 - DNA, 22 bp, Escherichia coli
  source 1..22: mol_type = other DNA
agtttcagcctttgcgagacgt

SEQ ID NO: 77 - DNA, 22 bp, Escherichia coli
  source 1..22: mol_type = other DNA
gatctgggggcaacacattgcc

SEQ ID NO: 78 - DNA, 20 bp, Escherichia coli
  source 1..20: mol_type = other DNA
gcagcggtttcagcggtaac

SEQ ID NO: 79 - DNA, 70 bp, Escherichia coli
  source 1..70: mol_type = other DNA
gcccgtagtccccagggaataataagaacagcatgtgggcgttattcatggtgtaggctggagctgcttc

SEQ ID NO: 80 - DNA, 70 bp, Escherichia coli
  source 1..70: mol_type = other DNA
acgcttgcgcgtcttatcaggcctacggtttacgcattacgttgcaacaacatatgaatatcctccttag

SEQ ID NO: 81 - DNA, 19 bp, Escherichia coli
  source 1..19: mol_type = other DNA
tcccgacgtctccaggtaa

SEQ ID NO: 82 - DNA, 20 bp, Escherichia coli
  source 1..20: mol_type = other DNA
ttgtctacgtagtggctcgc

SEQ ID NO: 83 - DNA, 20 bp, Escherichia coli
  source 1..20: mol_type = other DNA
gttgtgattggtgccggtgg

SEQ ID NO: 84 - DNA, 20 bp, Escherichia coli
  source 1..20: mol_type = other DNA
gcgtcatggattccgactct

SEQ ID NO: 85 - DNA, 20 bp, Escherichia coli
  source 1..20: mol_type = other DNA
tcgtccagccgaaagacttc

SEQ ID NO: 86 - DNA, 20 bp, Escherichia coli
  source 1..20: mol_type = other DNA
gtccagccattccccgttaa

SEQ ID NO: 87 - DNA, 24 bp, Escherichia coli
  source 1..24: mol_type = other DNA
gcaagatgctggttgccacgtccg

SEQ ID NO: 88 - DNA, 20 bp, Escherichia coli
  source 1..20: mol_type = other DNA
gcattgcaggtgtggatcgt

SEQ ID NO: 89 - DNA, 70 bp, Escherichia coli
  source 1..70: mol_type = other DNA
ttgcagcagcaggctggcgaaggtactgaagaacatcaggatgcctgatggtgtaggctggagctgcttc

SEQ ID NO: 90 - DNA, 70 bp, Escherichia coli
  source 1..70: mol_type = other DNA
gtcatagcggtaacaaaggttccctggggttagtggctgctgcgctcgtccatatgaatatcctccttag

SEQ ID NO: 91 - DNA, 24 bp, Escherichia coli
  source 1..24: mol_type = other DNA
ggtattttctccatcgcgggtatc

SEQ ID NO: 92 - DNA, 22 bp, Escherichia coli
  source 1..22: mol_type = other DNA
atgtagctcagtgcactgccaa

SEQ ID NO: 93 - DNA, 22 bp, Escherichia coli
  source 1..22: mol_type = other DNA
ctcggttattggcatttcaacg

SEQ ID NO: 94 - DNA, 22 bp, Escherichia coli
  source 1..22: mol_type = other DNA
catcaccctggcaagaaatggc